European Patent Application EP 4 218 816 A2, published August 2, 2023. Title: PHARMACEUTICAL COMPOSITION FOR USE IN PREVENTION AND/OR TREATMENT OF DISEASE THAT DEVELOPS OR PROGRESSES AS A RESULT OF DECREASE OR LOSS OF ACTIVITY OF BLOOD COAGULATION FACTOR VIII AND/OR ACTIVATED BLOOD COAGULATION FACTOR VIII. Applicant: CHUGAI SEIYAKU KABUSHIKI KAISHA. Application EP. The sequence listing filed with the application follows.

SEQUENCE LISTING (36 sequences)

SEQ ID NO: 1 - protein, 448 aa, synthetic construct
  REGION 1..448: note = synthesized
QVQLVESGGGLVQPGGSLRLSCAASGFTFSYYDMAWVRQAPGKGLEWVASISPSGGSTYYRHSVKGRFTVSRDNAKNSLYLQMNSLRAEDTAVYYCARRAGHNLGAGWYFDFWGQGTLVTVSSASTKGPSVFPLAPCSRSTSESTAALGCLVKDYFPEPVTVSWNSGALTSGVHTFPAVLQSSGLYSLSSVVTVPSSSLGTKTYTCNVDHKPSNTKVDKRVESKYGPPCPPCPAPEFLGGPSVFLFPPKPKDTLMISRTPEVTCVVVDVSQEDPEVQFNWYVDGVEVHNAKTKPREEQFNSTYRVVSVLTVLHQDWLNGKEYKCKVSNKGLPSSIEKTISKAKGQPREPQVCTLPPSQEEMTKNQVSLWCLVKGFYPSDIAVEWESNGQPENNYKTTPPVLDSDGSFFLYSRLTVDKSRWQEGNVFSCSVMHEALHNHYTQKSLSLSL

SEQ ID NO: 2 - protein, 448 aa, synthetic construct
  REGION 1..448: note = synthesized
QVQLVESGGGLVQPGGSLRLSCAASGFTFSYYDMAWVRQAPGKGLEWVASISPSGGSTYYRRSVKGRFTVSRDNAKNSLYLQMNSLRAEDTAVYYCARRAGHNLGAGWYFDFWGQGTLVTVSSASTKGPSVFPLAPCSRSTSESTAALGCLVKDYFPEPVTVSWNSGALTSGVHTFPAVLQSSGLYSLSSVVTVPSSSLGTKTYTCNVDHKPSNTKVDKRVESKYGPPCPPCPAPEFLGGPSVFLFPPKPKDTLMISRTPEVTCVVVDVSQEDPEVQFNWYVDGVEVHNAKTKPREEQFNSTYRVVSVLTVLHQDWLNGKEYKCKVSNKGLPSSIEKTISKAKGQPREPQVYTLPPSQKEMTKNQVSLTCLVKGFYPSDIAVEWESNGQPENNYKTTPPVLDSDGSFFLYSRLTVDKSRWQEGNVFSCSVMHEALHNHYTQKSLSLSL

SEQ ID NO: 3 - protein, 448 aa, synthetic construct
  REGION 1..448: note = synthesized
QVQLVESGGGLVQPGGSLRLSCAASGFTFSYYDMAWVRQAPGKGLEWVASISPSGGSTYYRRSVKGRFTVSRDNAKNSLYLQMNSLRAEDTAVYYCARRAGHNFGAGWYFDFWGQGTLVTVSSASTKGPSVFPLAPCSRSTSESTAALGCLVKDYFPEPVTVSWNSGALTSGVHTFPAVLQSSGLYSLSSVVTVPSSSLGTKTYTCNVDHKPSNTKVDKRVESKYGPPCPSCPAPEFLGGPSVFLFPPKPKDTLMISRTPEVTCVVVDVSQEDPEVQFNWYVDGVEVHNAKTKPREEQFNSTYRVVSVLTVLHQDWLNGKEYKCKVSNKGLPSSIEKTISKAKGQPREPQVYTLPPSQKEMTKNQVSLTCLVKGFYPSDIAVEWESNGQPENNYKTTPPVLDSDGSFFLYSRLTVDKSRWQEGNVFSCSVMHEALHNHYTQKSLSLSL

SEQ ID NO: 4 - protein, 444 aa, synthetic construct
  REGION 1..444: note = synthesized
QVQLVQSGSELKKPGASVKVSCKASGYTFTDNNMDWVRQAPGQGLEWMGDINTRSGGSIYNEEFQDRVIMTVDKSTGTAYMELSSLRSEDTAVYHCARRKSRGYHLDEWGEGTLVTVSSASTKGPSVFPLAPCSRSTSESTAALGCLVKDYFPEPVTVSWNSGALTSGVHTFPAVLQSSGLYSLSSVVTVPSSSLGTKTYTCNVDHKPSNTKVDKRVESKYGPPCPPCPAPEFLGGPSVFLFPPKPKDTLMISRTPEVTCVVVDVSQEDPEVQFNWYVDGVEVHNAKTKPREEQFNSTYRVVSVLTVLHQDWLNGKEYKCKVSNKGLPSSIEKTISKAKGQPREPQVYTLPPSQCEMTKNQVSLSCAVKGFYPSDIAVEWESNGQPENNYKTTPPVLDSDGSFFLVSRLTVDKSRWQEGNVFSCSVMHEALHNHYTQKSLSLSL

SEQ ID NO: 5 - protein, 444 aa, synthetic construct
  REGION 1..444: note = synthesized
QVQLVQSGSELKKPGASVKVSCKASGYTFTDNNMHWVRQAPGQGLEWMGDINTRSGGSIYNEEFQDRVIMTVDKSTDTAYMELSSLRSEDTAVYHCARRKSYGYHLDEWGEGTLVTVSSASTKGPSVFPLAPCSRSTSESTAALGCLVKDYFPEPVTVSWNSGALTSGVHTFPAVLQSSGLYSLSSVVTVPSSSLGTKTYTCNVDHKPSNTKVDKRVESKYGPPCPPCPAPEFLGGPSVFLFPPKPKDTLMISRTPEVTCVVVDVSQEDPEVQFNWYVDGVEVHNAKTKPREEQFNSTYRVVSVLTVLHQDWLNGKEYKCKVSNKGLPSSIEKTISKAKGQPREPQVYTLPPSQCEMTKNQVSLSCAVKGFYPSDIAVEWESNGQPENNYKTTPPVLDSDGSFFLVSRLTVDKSRWQEGNVFSCSVMHEALHNHYTQKSLSLSL

SEQ ID NO: 6 - protein, 444 aa, synthetic construct
  REGION 1..444: note = synthesized
QVQLVQSGSELKKPGASVKVSCKASGYTFTDNNMDWVRQAPGQGLEWMGDINTRSGGSIYNEEFQDRVIMTVDKSTDTAYMELSSLRSEDTAVYHCARRKSYGNHLDEWGEGTLVTVSSASTKGPSVFPLAPCSRSTSESTAALGCLVKDYFPEPVTVSWNSGALTSGVHTFPAVLQSSGLYSLSSVVTVPSSSLGTQTYTCNVDHKPSNTKVDKRVESKYGPPCPPCPAPEFLGGPSVFLFPPKPKDTLMISRTPEVTCVVVDVSQEDPEVQFNWYVDGVEVHNAKTKPREEQYNSTYRVVSVLTVLHQDWLNGKEYKCKVSNKGLPSSIEKTISKAKGQPREPQVYTLPPSQEEMTKNQVSLTCLVKGFYPSDIAVEWESNGQPENNYKTTPPVLDSDGSFFLYSKLTVDKSRWQEGNVFSCSVMHEALHNRYTQESLSLSP

SEQ ID NO: 7 - protein, 444 aa, synthetic construct
  REGION 1..444: note = synthesized
QVQLVQSGSELKKPGASVKVSCKASGYTFTDNNMDWVRQAPGQGLEWMGDINTKSGGSIYNEEFQDRVIMTVDKSTDTAYMELSSLRSEDTATYHCARRQSYGYHLDEWGEGTLVTVSSASTKGPSVFPLAPCSRSTSESTAALGCLVKDYFPEPVTVSWNSGALTSGVHTFPAVLQSSGLYSLSSVVTVPSSSLGTQTYTCNVDHKPSNTKVDKRVESKYGPPCPPCPAPEFLGGPSVFLFPPKPKDTLMISRTPEVTCVVVDVSQEDPEVQFNWYVDGVEVHNAKTKPREEQYNSTYRVVSVLTVLHQDWLNGKEYKCKVSNKGLPSSIEKTISKAKGQPREPQVYTLPPSQEEMTKNQVSLTCLVKGFYPSDIAVEWESNGQPENNYKTTPPVLDSDGSFFLYSKLTVDKSRWQEGNVFSCSVMHEALHNRYTQESLSLSP

SEQ ID NO: 8 - protein, 213 aa, synthetic construct
  REGION 1..213: note = synthesized
DIQMTQSPSSLSASVGDRVTITCKASQNIYKNLAWYQQKPGQAPKLLIYSASYRYSGVPDRFSGSRYGTDFTLTISSLQPEDLATYYCQQYYSGLTFGGGTKVEIKRTVAAPSVFIFPPSDEQLKSGTASVVCLLNNFYPREAKVQWKVDNALQSGNSQESVTEQDSKDSTYSLSSTLTLSKADYEKHKVYACEVTHQGLSSPVTKSFNRGEC

SEQ ID NO: 9 - protein, 214 aa, synthetic construct
  REGION 1..214: note = synthesized
DIQMTQSPSSLSASVGDRVTITCKASQNIYKNLAWYQQKPGQAPKLLIYSASYRYSGVPDRFSGSRYGTDFTLTISSLQPEDLATYYCQQYYSPPLTFGGGTKVEIKRTVAAPSVFIFPPSDEQLKSGTASVVCLLNNFYPREAKVQWKVDNALQSGNSQESVTEQDSKDSTYSLSSTLTLSKADYEKHKVYACEVTHQGLSSPVTKSFNRGEC

SEQ ID NO: 10 - protein, 448 aa, synthetic construct
  REGION 1..448: note = synthesized
QVQLVESGGGLVQPGGSLRLSCAASGFTFSYYDMAWVRQAPGKGLEWVASISPSGGSTYYRRSVKGRFTVSRDNAKNSLYLQMNSLRAEDTAVYYCARRAGHNFGAGWYFDFWGQGTLVTVSSASTKGPSVFPLAPCSRSTSESTAALGCLVKDYFPEPVTVSWNSGALTSGVHTFPAVLQSSGLYSLSSVVTVPSSSLGTKTYTCNVDHKPSNTKVDKRVESKYGPPCPPCPAPEFLGGPSVFLFPPKPKDTLMISRTPEVTCVVVDVSQEDPEVQFNWYVDGVEVHNAKTKPREEQFNSTYRVVSVLTVLHQDWLNGKEYKCKVSNKGLPSSIEKTISKAKGQPREPQVYTLPPSQKEMTKNQVSLTCLVKGFYPSDIAVEWESNGQPENNYKTTPPVLDSDGSFFLYSRLTVDKSRWQEGNVFSCSVMHEALHNHYTQKSLSLSL

SEQ ID NO: 11 - protein, 448 aa, synthetic construct
  REGION 1..448: note = synthesized
QVQLVESGGGLVQPGGSLRLSCAASGFTFSYYDMAWVRQAPGKGLEWVASISPSGGSTYYRRSVKGRFTVSRDNAKNSLYLQMNSLRAEDTAVYYCARRAGHNYGAGWYFDYWGQGTLVTVSSASTKGPSVFPLAPCSRSTSESTAALGCLVKDYFPEPVTVSWNSGALTSGVHTFPAVLQSSGLYSLSSVVTVPSSSLGTKTYTCNVDHKPSNTKVDKRVESKYGPPCPPCPAPEFLGGPSVFLFPPKPKDTLMISRTPEVTCVVVDVSQEDPEVQFNWYVDGVEVHNAKTKPREEQFNSTYRVVSVLTVLHQDWLNGKEYKCKVSNKGLPSSIEKTISKAKGQPREPQVCTLPPSQEEMTKNQVSLWCLVKGFYPSDIAVEWESNGQPENNYKTTPPVLDSDGSFFLYSRLTVDKSRWQEGNVFSCSVMHEALHNHYTQKSLSLSL

SEQ ID NO: 12 - protein, 448 aa, synthetic construct
  REGION 1..448: note = synthesized
QVQLVESGGGLVQPGGSLRLSCAASGFTFSYYDINWVRQAPGKGLEWVASISPSGGSTYYRRSVKGRFTISRDNAKNSLYLQMNSLRAEDTAVYYCATRAGHNYGAGWYFDYWGQGTLVTVSSASTKGPSVFPLAPCSRSTSESTAALGCLVKDYFPEPVTVSWNSGALTSGVHTFPAVLQSSGLYSLSSVVTVPSSSLGTKTYTCNVDHKPSNTKVDKRVESKYGPPCPPCPAPEFLGGPSVFLFPPKPKDTLMISRTPEVTCVVVDVSQEDPEVQFNWYVDGVEVHNAKTKPREEQFNSTYRVVSVLTVLHQDWLNGKEYKCKVSNKGLPSSIEKTISKAKGQPREPQVCTLPPSQEEMTKNQVSLWCLVKGFYPSDIAVEWESNGQPENNYKTTPPVLDSDGSFFLYSRLTVDKSRWQEGNVFSCSVMHEALHNHYTQKSLSLSL

SEQ ID NO: 13 - protein, 448 aa, synthetic construct
  REGION 1..448: note = synthesized
QVQLVESGGGLVQPGGSLRLSCAASGFTFSYYDINWVRQAPGKGLEWVSSISPSGQSTYYRREVKGRFTISRDNSKNTLYLQMNSLRAEDTAVYYCARRSGHNYGGGWYFDYWGQGTLVTVSSASTKGPSVFPLAPCSRSTSESTAALGCLVKDYFPEPVTVSWNSGALTSGVHTFPAVLQSSGLYSLSSVVTVPSSSLGTQTYTCNVDHKPSNTKVDKRVESKYGPPCPPCPAPEFLGGPSVFLFPPKPKDTLMISRTPEVTCVVVDVSQEDPEVQFNWYVDGVEVHNAKTKPREEQYNSTYRVVSVLTVLHQDWLNGKEYKCKVSNKGLPSSIEKTISKAKGQPREPQVYTLPPSQKEMTKNQVSLTCLVKGFYPSDIAVEWESNGQPENNYKTTPPVLDSDGSFFLYSKLTVDKSRWQEGNVFSCSVMHEALHNHYTQKSLSLSL

SEQ ID NO: 14 - protein, 448 aa, synthetic construct
  REGION 1..448: note = synthesized
QVQLVESGGGLVQPGGSLRLSCAASGFTFSYYDIQWVRQAPGKGLEWVSSISPSGQSTYYRREVKGRFTISRDNSKNTLYLQMNSLRAEDTAVYYCARRSGHNYGGGWYFDYWGQGTLVTVSSASTKGPSVFPLAPCSRSTSESTAALGCLVKDYFPEPVTVSWNSGALTSGVHTFPAVLQSSGLYSLSSVVTVPSSSLGTKTYTCNVDHKPSNTKVDKRVESKYGPPCPPCPAPEFLGGPSVFLFPPKPKDTLMISRTPEVTCVVVDVSQEDPEVQFNWYVDGVEVHNAKTKPREEQFNSTYRVVSVLTVLHQDWLNGKEYKCKVSNKGLPSSIEKTISKAKGQPREPQVCTLPPSQEEMTKNQVSLWCLVKGFYPSDIAVEWESNGQPENNYKTTPPVLDSDGSFFLYSRLTVDKSRWQEGNVFSCSVMHEALHNHYTQKSLSLSL

SEQ ID NO: 15 - protein, 448 aa, synthetic construct
  REGION 1..448: note = synthesized
QVQLVESGGGLVQPGGSLRLSCAASGFTFSYYDIQWVRQAPGKGLEWVSSISPSGQSTYYRREVKGRFTISRDNSKNTLYLQMNSLRAEDTAVYYCARRSGHNYGGGWYFDYWGQGTLVTVSSASTKGPSVFPLAPCSRSTSESTAALGCLVKDYFPEPVTVSWNSGALTSGVHTFPAVLQSSGLYSLSSVVTVPSSSLGTQTYTCNVDHKPSNTKVDKRVESKYGPPCPPCPAPEFLGGPSVFLFPPKPKDTLMISRTPEVTCVVVDVSQEDPEVQFNWYVDGVEVHNAKTKPREEQYNSTYRVVSVLTVLHQDWLNGKEYKCKVSNKGLPSSIEKTISKAKGQPREPQVYTLPPSQKEMTKNQVSLTCLVKGFYPSDIAVEWESNGQPENNYKTTPPVLDSDGSFFLYSKLTVDKSRWQEGNVFSCSVMHEALHNHYTQKSLSLSP

SEQ ID NO: 16 - protein, 448 aa, synthetic construct
  REGION 1..448: note = synthesized
QVQLVESGGGLVQPGGSLRLSCAASGFTFSYYDISWVRQAPGKGLEWVSSISPSGQSTYYRREVKGRFTISRDNSKNTLYLQMNSLRAEDTAVYYCARRSGHNFGGGWYFDYWGQGTLVTVSSASTKGPSVFPLAPCSRSTSESTAALGCLVKDYFPEPVTVSWNSGALTSGVHTFPAVLQSSGLYSLSSVVTVPSSSLGTKTYTCNVDHKPSNTKVDKRVESKYGPPCPPCPAPEFLGGPSVFLFPPKPKDTLMISRTPEVTCVVVDVSQEDPEVQFNWYVDGVEVHNAKTKPREEQFNSTYRVVSVLTVLHQDWLNGKEYKCKVSNKGLPSSIEKTISKAKGQPREPQVCTLPPSQEEMTKNQVSLWCLVKGFYPSDIAVEWESNGQPENNYKTTPPVLDSDGSFFLYSRLTVDKSRWQEGNVFSCSVMHEALHNHYTQKSLSLSL

SEQ ID NO: 17 - protein, 448 aa, synthetic construct
  REGION 1..448: note = synthesized
QVQLVESGGGLVQPGGSLRLSCAASGFTFSYYDIQWVRQAPGKGLEWVSSISPSGQSTYYRREVKGRFTISRDNSKNTLYLQMNSLRAEDTAVYYCARRSGKSYGGGWYFDYWGQGTLVTVSSASTKGPSVFPLAPCSRSTSESTAALGCLVKDYFPEPVTVSWNSGALTSGVHTFPAVLQSSGLYSLSSVVTVPSSSLGTQTYTCNVDHKPSNTKVDKRVESKYGPPCPPCPAPEFLGGPSVFLFPPKPKDTLMISRTPEVTCVVVDVSQEDPEVQFNWYVDGVEVHNAKTKPREEQYNSTYRVVSVLTVLHQDWLNGKEYKCKVSNKGLPSSIEKTISKAKGQPREPQVYTLPPSQKEMTKNQVSLTCLVKGFYPSDIAVEWESNGQPENNYKTTPPVLDSDGSFFLYSKLTVDKSRWQEGNVFSCSVMHEALHNHYTQKSLSLSL

SEQ ID NO: 18 - protein, 448 aa, synthetic construct
  REGION 1..448: note = synthesized
QVQLVESGGGLVQPGGSLRLSCAASGFTFSYYDIQWVRQAPGKGLEWVSSISPSGQSTYYRREVKGRFTISRDNSKNTLYLQMNSLRAEDTAVYYCARRSGREYGGGWYFDYWGQGTLVTVSSASTKGPSVFPLAPCSRSTSESTAALGCLVKDYFPEPVTVSWNSGALTSGVHTFPAVLQSSGLYSLSSVVTVPSSSLGTQTYTCNVDHKPSNTKVDKRVESKYGPPCPPCPAPEFLGGPSVFLFPPKPKDTLMISRTPEVTCVVVDVSQEDPEVQFNWYVDGVEVHNAKTKPREEQYNSTYRVVSVLTVLHQDWLNGKEYKCKVSNKGLPSSIEKTISKAKGQPREPQVYTLPPSQKEMTKNQVSLTCLVKGFYPSDIAVEWESNGQPENNYKTTPPVLDSDGSFFLYSKLTVDKSRWQEGNVFSCSVMHEALHNRYTQKSLSLSP

SEQ ID NO: 19 - protein, 448 aa, synthetic construct
  REGION 1..448: note = synthesized
QVQLVESGGGLVQPGGSLRLSCAASGFTFSYYDIQWVRQAPGKGLEWVSSISPSGQSTYYRREVKGRFTISRDNSKNTLYLQMNSLRAEDTAVYYCARRTGREYGGGWYFDYWGQGTLVTVSSASTKGPSVFPLAPCSRSTSESTAALGCLVKDYFPEPVTVSWNSGALTSGVHTFPAVLQSSGLYSLSSVVTVPSSSLGTQTYTCNVDHKPSNTKVDKRVESKYGPPCPPCPAPEFLGGPSVFLFPPKPKDTLMISRTPEVTCVVVDVSQEDPEVQFNWYVDGVEVHNAKTKPREEQYNSTYRVVSVLTVLHQDWLNGKEYKCKVSNKGLPSSIEKTISKAKGQPREPQVYTLPPSQKEMTKNQVSLTCLVKGFYPSDIAVEWESNGQPENNYKTTPPVLDSDGSFFLYSKLTVDKSRWQEGNVFSCSVMHEALHNHYTQKSLSLSP

SEQ ID NO: 20 - protein, 448 aa, synthetic construct
  REGION 1..448: note = synthesized
QVQLVESGGGLVQPGGSLRLSCAASGFTFSYYDIQWVRQAPGKGLEWVSSISPSGQSTYYRREVKGRFTISRDNSKNTLYLQMNSLRAEDTAVYYCARRTGREYGGGWYFDYWGQGTLVTVSSASTKGPSVFPLAPCSRSTSESTAALGCLVKDYFPEPVTVSWNSGALTSGVHTFPAVLQSSGLYSLSSVVTVPSSSLGTQTYTCNVDHKPSNTKVDKRVESKYGPPCPPCPAPEFLGGPSVFLFPPKPKDTLMISRTPEVTCVVVDVSQEDPEVQFNWYVDGVEVHNAKTKPREEQYNSTYRVVSVLTVLHQDWLNGKEYKCKVSNKGLPSSIEKTISKAKGQPREPQVYTLPPSQKEMTKNQVSLTCLVKGFYPSDIAVEWESNGQPENNYKTTPPVLDSDGSFFLYSKLTVDKSRWQEGNVFSCSVMHEALHNRYTQKSLSLSP

SEQ ID NO: 21 - protein, 444 aa, synthetic construct
  REGION 1..444: note = synthesized
QVQLVQSGSELKKPGASVKVSCKASGYTFTDNNMDWVRQAPGQGLEWMGDINTRSGGSIYNEEFQDRVIMTVDKSTGTAYMELSSLRSEDTAVYYCARRKSYGYHLDEWGEGTLVTVSSASTKGPSVFPLAPCSRSTSESTAALGCLVKDYFPEPVTVSWNSGALTSGVHTFPAVLQSSGLYSLSSVVTVPSSSLGTKTYTCNVDHKPSNTKVDKRVESKYGPPCPPCPAPEFLGGPSVFLFPPKPKDTLMISRTPEVTCVVVDVSQEDPEVQFNWYVDGVEVHNAKTKPREEQFNSTYRVVSVLTVLHQDWLNGKEYKCKVSNKGLPSSIEKTISKAKGQPREPQVYTLPPSQCEMTKNQVSLSCAVKGFYPSDIAVEWESNGQPENNYKTTPPVLDSDGSFFLVSRLTVDKSRWQEGNVFSCSVMHEALHNHYTQKSLSLSL

SEQ ID NO: 22 - protein, 444 aa, synthetic construct
  REGION 1..444: note = synthesized
QVQLVQSGSELKKPGASVKVSCKASGYTFTDNNMDWVRQAPGQGLEWMGDINTRSGGSIYNEEFQDRVIMTVDKSTGTAYMELSSLRSEDTAVYHCARRKSYGYYLDEWGEGTLVTVSSASTKGPSVFPLAPCSRSTSESTAALGCLVKDYFPEPVTVSWNSGALTSGVHTFPAVLQSSGLYSLSSVVTVPSSSLGTQTYTCNVDHKPSNTKVDKRVESKYGPPCPPCPAPEFLGGPSVFLFPPKPKDTLMISRTPEVTCVVVDVSQEDPEVQFNWYVDGVEVHNAKTKPREEQYNSTYRVVSVLTVLHQDWLNGKEYKCKVSNKGLPSSIEKTISKAKGQPREPQVYTLPPSQEEMTKNQVSLTCLVKGFYPSDIAVEWESNGQPENNYKTTPPVLDSDGSFFLYSKLTVDKSRWQEGNVFSCSVMHEALHNRYTQESLSLSP

SEQ ID NO: 23 - protein, 444 aa, synthetic construct
  REGION 1..444: note = synthesized
QVQLVQSGSELKKPGASVKVSCKASGYTFTDNNMDWVRQAPGQGLEWMGDINTRSGGSIYNEEFQDRVIMTVDKSTDTAYMELSSLRSEDTAVYHCARRKSYGYYLDEWGEGTLVTVSSASTKGPSVFPLAPCSRSTSESTAALGCLVKDYFPEPVTVSWNSGALTSGVHTFPAVLQSSGLYSLSSVVTVPSSSLGTQTYTCNVDHKPSNTKVDKRVESKYGPPCPPCPAPEFLGGPSVFLFPPKPKDTLMISRTPEVTCVVVDVSQEDPEVQFNWYVDGVEVHNAKTKPREEQYNSTYRVVSVLTVLHQDWLNGKEYKCKVSNKGLPSSIEKTISKAKGQPREPQVYTLPPSQEEMTKNQVSLTCLVKGFYPSDIAVEWESNGQPENNYKTTPPVLDSDGSFFLYSKLTVDKSRWQEGNVFSCSVMHEALHNRYTQESLSLSP

SEQ ID NO: 24 - protein, 444 aa, synthetic construct
  REGION 1..444: note = synthesized
QVQLVQSGSELKKPGASVKVSCKASGYTFTDNNMDWVRQAPGQGLEWMGDINTRSGGSIYNEEFQDRVIMTVDKSTDTAYMELSSLRSEDTATYHCARRKSYGYYLDEWGEGTLVTVSSASTKGPSVFPLAPCSRSTSESTAALGCLVKDYFPEPVTVSWNSGALTSGVHTFPAVLQSSGLYSLSSVVTVPSSSLGTQTYTCNVDHKPSNTKVDKRVESKYGPPCPPCPAPEFLGGPSVFLFPPKPKDTLMISRTPEVTCVVVDVSQEDPEVQFNWYVDGVEVHNAKTKPREEQYNSTYRVVSVLTVLHQDWLNGKEYKCKVSNKGLPSSIEKTISKAKGQPREPQVYTLPPSQEEMTKNQVSLTCLVKGFYPSDIAVEWESNGQPENNYKTTPPVLDSDGSFFLYSKLTVDKSRWQEGNVFSCSVMHEALHNRYTQESLSLSP

SEQ ID NO: 25 - protein, 444 aa, synthetic construct
  REGION 1..444: note = synthesized
QVQLVQSGSELKKPGASVKVSCKASGYTFTDNNMDWVRQAPGQGLEWMGDINTRSGGSIYNEEFQDRVIMTVDKSTDTAYMELSSLRSEDTATYHCARRKSYGYYLDEWGEGTLVTVSSASTKGPSVFPLAPCSRSTSESTAALGCLVKDYFPEPVTVSWNSGALTSGVHTFPAVLQSSGLYSLSSVVTVPSSSLGTQTYTCNVDHKPSNTKVDKRVESKYGPPCPPCPAPEFLGGPSVFLFPPKPKDTLMISRTPEVTCVVVDVSQEDPEVQFNWYVDGVEVHNAKTKPREEQYNSTYRVVSVLTVLHQDWLNGKEYKCKVSNKGLPSSIEKTISKAKGQPREPQVYTLPPSQEEMTKNQVSLTCLVKGFYPSDIAVEWESNGQPENNYKTTPPVLDSDGSFFLYSKLTVDKSRWQEGNVFSCSVMHEALHNHYTQESLSLSP

SEQ ID NO: 26 - protein, 444 aa, synthetic construct
  REGION 1..444: note = synthesized
QVQLVQSGSELKKPGASVKVSCKASGYTFTDNNMDWVRQAPGQGLEWMGDINTRSGGSIYNEEFQDRVIMTVDTSTDTAYMELSSLRSEDTATYHCARRKSYGYHLDEWGEGTLVTVSSASTKGPSVFPLAPCSRSTSESTAALGCLVKDYFPEPVTVSWNSGALTSGVHTFPAVLQSSGLYSLSSVVTVPSSSLGTQTYTCNVDHKPSNTKVDKRVESKYGPPCPPCPAPEFLGGPSVFLFPPKPKDTLMISRTPEVTCVVVDVSQEDPEVQFNWYVDGVEVHNAKTKPREEQYNSTYRVVSVLTVLHQDWLNGKEYKCKVSNKGLPSSIEKTISKAKGQPREPQVYTLPPSQEEMTKNQVSLTCLVKGFYPSDIAVEWESNGQPENNYKTTPPVLDSDGSFFLYSKLTVDKSRWQEGNVFSCSVMHEALHNHYTQESLSLSP

SEQ ID NO: 27 - protein, 444 aa, synthetic construct
  REGION 1..444: note = synthesized
QVQLVQSGSELKKPGASVKVSCKASGYTFTDNNMDWVRQAPGQGLEWMGDINTRSGGSIYNEEFQDRVIMTVDKSTDTAYMELSSLRSEDTATYHCARRKSYGYHLDEWGEGTLVTVSSASTKGPSVFPLAPCSRSTSESTAALGCLVKDYFPEPVTVSWNSGALTSGVHTFPAVLQSSGLYSLSSVVTVPSSSLGTQTYTCNVDHKPSNTKVDKRVESKYGPPCPPCPAPEFLGGPSVFLFPPKPKDTLMISRTPEVTCVVVDVSQEDPEVQFNWYVDGVEVHNAKTKPREEQYNSTYRVVSVLTVLHQDWLNGKEYKCKVSNKGLPSSIEKTISKAKGQPREPQVYTLPPSQEEMTKNQVSLTCLVKGFYPSDIAVEWESNGQPENNYKTTPPVLDSDGSFFLYSKLTVDKSRWQEGNVFSCSVMHEALHNRYTQESLSLSP

SEQ ID NO: 28 - protein, 214 aa, synthetic construct
  REGION 1..214: note = synthesized
DIQMTQSPSSLSASVGDRVTITCKASKNIERNLAWYQQKPGQAPRLLIYRASRKESGVPDRFSGSRYGTDFTLTISSLQPEDIATYYCQQYSSPPLTFGGGTKVEIKRTVAAPSVFIFPPSDEQLKSGTASVVCLLNNFYPREAKVQWKVDNALQSGNSQESVTEQDSKDSTYSLSSTLTLSKADYEKHKVYACEVTHQGLSSPVTKSFNRGEC

SEQ ID NO: 29 - protein, 214 aa, synthetic construct
  REGION 1..214: note = synthesized
DIQMTQSPSSLSASVGDRVTITCKASRNIERNLAWYQQKPGQAPELLIYRADRKESGVPDRFSGSRYGTDFTLTISSLQPEDIATYYCQQYSSPPLTFGGGTKVEIKRTVAAPSVFIFPPSDEQLKSGTASVVCLLNNFYPREAKVQWKVDNALQSGNSQESVTEQDSKDSTYSLSSTLTLSKADYEKHKVYACEVTHQGLSSPVTKSFNRGEC

SEQ ID NO: 30 - protein, 214 aa, synthetic construct
  REGION 1..214: note = synthesized
DIQMTQSPSSLSASVGDRVTITCKASRNIERNLAWYQQKPGQAPELLIYQASRKESGVPDRFSGSRYGTDFTLTISSLQPEDIATYYCQQYSSPPLTFGGGTKVEIKRTVAAPSVFIFPPSDEQLKSGTASVVCLLNNFYPREAKVQWKVDNALQSGNSQESVTEQDSKDSTYSLSSTLTLSKADYEKHKVYACEVTHQGLSSPVTKSFNRGEC

SEQ ID NO: 31 - protein, 214 aa, synthetic construct
  REGION 1..214: note = synthesized
DIQMTQSPSSLSASVGDRVTITCKASRNIERQLAWYQQKPGQAPELLIYQASRKESGVPDRFSGSRYGTDFTLTISSLQPEDIATYYCQQYSSPPLTFGGGTKVEIKRTVAAPSVFIFPPSDEQLKSGTASVVCLLNNFYPREAKVQWKVDNALQSGNSQESVTEQDSKDSTYSLSSTLTLSKADYEKHKVYACEVTHQGLSSPVTKSFNRGEC

SEQ ID NO: 32 - protein, 214 aa, synthetic construct
  REGION 1..214: note = synthesized
DIQMTQSPSSLSASVGDRVTITCKASRNIERQLAWYQQKPGQAPELLIYQASRKESGVPDRFSGSRYGTDFTLTISSLQPEDIATYYCQQYSDPPLTFGGGTKVEIKRTVAAPSVFIFPPSDEQLKSGTASVVCLLNNFYPREAKVQWKVDNALQSGNSQESVTEQDSKDSTYSLSSTLTLSKADYEKHKVYACEVTHQGLSSPVTKSFNRGEC

SEQ ID NO: 33 - protein, 214 aa, synthetic construct
  REGION 1..214: note = synthesized
DIQMTQSPSSLSASVGDRVTITCKASRNIERQLAWYQQKPGQAPELLIYRASRKESGVPDRFSGSRYGTDFTLTISSLQPEDIATYYCQQYSDPPLTFGGGTKVEIKRTVAAPSVFIFPPSDEQLKSGTASVVCLLNNFYPREAKVQWKVDNALQSGNSQESVTEQDSKDSTYSLSSTLTLSKADYEKHKVYACEVTHQGLSSPVTKSFNRGEC

SEQ ID NO: 34 - protein, 214 aa, synthetic construct
  REGION 1..214: note = synthesized
DIQMTQSPSSLSASVGDRVTITCKASRNIERQLAWYQQKPGQAPELLIYRADRKESGVPDRFSGSRYGTDFTLTISSLQPEDIATYYCQQYSDPPLTFGGGTKVEIKRTVAAPSVFIFPPSDEQLKSGTASVVCLLNNFYPREAKVQWKVDNALQSGNSQESVTEQDSKDSTYSLSSTLTLSKADYEKHKVYACEVTHQGLSSPVTKSFNRGEC

SEQ ID NO: 35 - protein, 444 aa, synthetic construct
  REGION 1..444: note = synthesized
QVQLVQSGSELKKPGASVKVSCKASGYTFTDNNMDWVRQAPGQGLEWMGDINTRSGGSIYNEEFQDRVTMTIDKSTGTAYMELSSLRSEDTAVYYCARRRSYGYYHDEWGEGTLVTVSSASTKGPSVFPLAPCSRSTSESTAALGCLVKDYFPEPVTVSWNSGALTSGVHTFPAVLQSSGLYSLSSVVTVPSSSLGTKTYTCNVDHKPSNTKVDKRVESKYGPPCPPCPAPEFLGGPSVFLFPPKPKDTLMISRTPEVTCVVVDVSQEDPEVQFNWYVDGVEVHNAKTKPREEQFNSTYRVVSVLTVLHQDWLNGKEYKCKVSNKGLPSSIEKTISKAKGQPREPQVYTLPPSQCEMTKNQVSLSCAVKGFYPSDIAVEWESNGQPENNYKTTPPVLDSDGSFFLVSRLTVDKSRWQEGNVFSCSVMHEALHNHYTQKSLSLSL

SEQ ID NO: 36 - protein, 214 aa, synthetic construct
  REGION 1..214: note = synthesized
DIQMTQSPSSLSASVGDRVTITCKASRNIERNLAWYQQKPGQAPELLIYSASRKESGVPDRFSGSRYGTDFTLTISSLQPEDLATYYCQQYYSPPLTFGGGTKVEIKRTVAAPSVFIFPPSDEQLKSGTASVVCLLNNFYPREAKVQWKVDNALQSGNSQESVTEQDSKDSTYSLSSTLTLSKADYEKHKVYACEVTHQGLSSPVTKSFNRGEC